European Patent Application EP 4 527 385 A1, published March 26, 2025. Title: IL-6 and/or IL-1beta suppressor. Applicant: AGC株式会社. Application JP. The sequence listing filed with the application follows.

SEQUENCE LISTING (4 sequences)

SEQ ID NO: 1 - DNA, 21 bp, synthetic construct
  misc_feature 1..21: note = primer
  source 1..21: mol_type = other DNA
agcgatgatgcactgtcagaa

SEQ ID NO: 2 - DNA, 21 bp, synthetic construct
  misc_feature 1..21: note = primer
  source 1..21: mol_type = other DNA
aacggaactccagaagaccag

SEQ ID NO: 3 - DNA, 25 bp, synthetic construct
  misc_feature 1..25: note = primer
  source 1..25: mol_type = other DNA
ccctgaactcaactgtgaaatagca

SEQ ID NO: 4 - DNA, 20 bp, synthetic construct
  misc_feature 1..20: note = primer
  source 1..20: mol_type = other DNA
cccaagtcaagggcttggaa